European Patent Application EP 4 560 018 A1, published May 28, 2025. Title: METHOD FOR THE GENERATION OF A CDNA LIBRARY FROM AN RNA SAMPLE. Applicant: Servicio Andaluz de Salud. Application EP. The sequence listing filed with the application follows.

SEQUENCE LISTING (60 sequences)

SEQ ID NO: 1 - DNA, 23 bp, synthetic construct
  source 1..23: mol_type = other DNA
aaaaaaaaaaaaaaaaaaaaaaa

SEQ ID NO: 2 - DNA, 21 bp, synthetic construct
  source 1..21: mol_type = other DNA
aaaaaaaaaaaaaaaaaaaaa

SEQ ID NO: 3 - DNA, 21 bp, synthetic construct
  source 1..21: mol_type = other DNA
ttttttttttttttttttttt

SEQ ID NO: 4 - DNA, 21 bp, synthetic construct
  source 1..21: mol_type = other DNA
aaaaaaaaaaaaaaaaaaaaa

SEQ ID NO: 5 - DNA, 21 bp, synthetic construct
  source 1..21: mol_type = other DNA
ttttttttttttttttttttt

SEQ ID NO: 6 - DNA, 26 bp, synthetic construct
  source 1..26: mol_type = other DNA
aaaaaaaaaaaaaaaaaaaaaaaaaa

SEQ ID NO: 7 - DNA, 20 bp, synthetic construct
  source 1..20: mol_type = other DNA
tttttttttttttttttttt

SEQ ID NO: 8 - DNA, 20 bp, synthetic construct
  source 1..20: mol_type = other DNA
tttttttttttttttttttt

SEQ ID NO: 9 - DNA, 20 bp, synthetic construct
  source 1..20: mol_type = other DNA
tttttttttttttttttttt

SEQ ID NO: 10 - DNA, 20 bp, synthetic construct
  source 1..20: mol_type = other DNA
tttttttttttttttttttt

SEQ ID NO: 11 - DNA, 20 bp, synthetic construct
  source 1..20: mol_type = other DNA
tttttttttttttttttttt

SEQ ID NO: 12 - skipped

SEQ ID NO: 13 - DNA, 18 bp, synthetic construct
  source 1..18: mol_type = other DNA
tttttttttttttttttt

SEQ ID NO: 14 - DNA, 18 bp, synthetic construct
  source 1..18: mol_type = other DNA
tttttttttttttttttt

SEQ ID NO: 15 - DNA, 18 bp, synthetic construct
  source 1..18: mol_type = other DNA
tttttttttttttttttt

SEQ ID NO: 16 - DNA, 18 bp, synthetic construct
  source 1..18: mol_type = other DNA
tttttttttttttttttt

SEQ ID NO: 17-18 - skipped (2 entries)

SEQ ID NO: 19 - DNA, 169 bp, synthetic construct
  source 1..169: mol_type = other DNA
tcagacgtgtgctcttccgatccccccccccccccccctggcagtgtcttagctggttgtaaaaaaaaaaaaaaaaaaaaaaagatcggaagagcgtcgtgtagggaaagagtgtagatctcggtggtcgccgtatcattaatcactagtgcggccgcctgcaggtcga

SEQ ID NO: 20 - DNA, 168 bp, synthetic construct
  source 1..168: mol_type = other DNA
cgtgtgctcttccgatcccccccccccccccaaatttctgtttcaaactgaaaaaaaaaaaaaaaaaaaaaaaaaaaaaagatcggaagagcgtcgtgtagggaaagagtgtagatctcggtggtcgccgtatcattaatcactagtgcggccgcctgcaggtcgacc

SEQ ID NO: 21 - RNA, 41 nt, synthetic construct
  source 1..41: mol_type = other RNA
agaagcagagatctcacacaaaaaaaaaaaaaaaaaaaaaa

SEQ ID NO: 22 - RNA, 23 nt, synthetic construct
  source 1..23: mol_type = other RNA
tatggctttttattcctatgtga

SEQ ID NO: 23 - RNA, 23 nt, synthetic construct
  source 1..23: mol_type = other RNA
tatggcttttcattcctatgtga

SEQ ID NO: 24 - RNA, 21 nt, synthetic construct
  source 1..21: mol_type = other RNA
ttcaagtaattcaggataggt

SEQ ID NO: 25 - RNA, 22 nt, synthetic construct
  source 1..22: mol_type = other RNA
tggcagtgtcttagctggttgt

SEQ ID NO: 26 - RNA, 23 nt, synthetic construct
  source 1..23: mol_type = other RNA
taggcagtgtcattagctgattg

SEQ ID NO: 27 - RNA, 23 nt, synthetic construct
  source 1..23: mol_type = other RNA
aggcagtgtagttagctgattgc

SEQ ID NO: 28 - RNA, 23 nt, synthetic construct
  source 1..23: mol_type = other RNA
gtccagttttcccaggaatccct

SEQ ID NO: 29 - RNA, 31 nt, synthetic construct
  source 1..31: mol_type = other RNA
  modified_base 26..27: mod_base = OTHER; note = Thymine
  modified_base 29: mod_base = OTHER; note = Thymine
tccctgagaccctaacttgtgaaacttgtga

SEQ ID NO: 30 - RNA, 22 nt, synthetic construct
  source 1..22: mol_type = other RNA
aaaagctgggttgagagggcga

SEQ ID NO: 31 - RNA, 23 nt, synthetic construct
  source 1..23: mol_type = other RNA
atcacattgccagggattaccac

SEQ ID NO: 32 - RNA, 23 nt, synthetic construct
  source 1..23: mol_type = other RNA
caaagtgcttacagtgcaggtag

SEQ ID NO: 33 - RNA, 23 nt, synthetic construct
  source 1..23: mol_type = other RNA
taaggtgcatctagtgcagatag

SEQ ID NO: 34 - RNA, 23 nt, synthetic construct
  source 1..23: mol_type = other RNA
taaagtgcttatagtgcaggtag

SEQ ID NO: 35 - RNA, 22 nt, synthetic construct
  source 1..22: mol_type = other RNA
tagcttatcagactgatgttga

SEQ ID NO: 36 - RNA, 21 nt, synthetic construct
  source 1..21: mol_type = other RNA
atcacattgccagggatttcc

SEQ ID NO: 37 - RNA, 22 nt, synthetic construct
  source 1..22: mol_type = other RNA
tggctcagttcagcaggaacag

SEQ ID NO: 38 - RNA, 22 nt, synthetic construct
  source 1..22: mol_type = other RNA
tagcaccatttgaaatcggtta

SEQ ID NO: 39 - RNA, 24 nt, synthetic construct
  source 1..24: mol_type = other RNA
tccctgagaccctttaacctgtga

SEQ ID NO: 40 - RNA, 22 nt, synthetic construct
  source 1..22: mol_type = other RNA
cagtgcaatgttaaaagggcat

SEQ ID NO: 41 - RNA, 22 nt, synthetic construct
  source 1..22: mol_type = other RNA
tctcccaacccttgtaccagtg

SEQ ID NO: 42 - RNA, 23 nt, synthetic construct
  source 1..23: mol_type = other RNA
taatactgccgggtaatgatgga

SEQ ID NO: 43 - RNA, 22 nt, synthetic construct
  source 1..22: mol_type = other RNA
ctgtgcgtgtgacagcggctga

SEQ ID NO: 44 - RNA, 23 nt, synthetic construct
  source 1..23: mol_type = other RNA
agctacattgtctgctgggtttc

SEQ ID NO: 45 - RNA, 23 nt, synthetic construct
  source 1..23: mol_type = other RNA
cagtgcaatagtattgtcaaagc

SEQ ID NO: 46 - RNA, 22 nt, synthetic construct
  source 1..22: mol_type = other RNA
taatgcccctaaaaatccttat

SEQ ID NO: 47 - RNA, 23 nt, synthetic construct
  source 1..23: mol_type = other RNA
tagtgcaatattgcttatagggt

SEQ ID NO: 48 - RNA, 22 nt, synthetic construct
  source 1..22: mol_type = other RNA
ggtggcccggccgtgcctgagg

SEQ ID NO: 49 - RNA, 24 nt, synthetic construct
  source 1..24: mol_type = other RNA
gaagtcctcttccaactcctgttg

SEQ ID NO: 50 - RNA, 24 nt, synthetic construct
  source 1..24: mol_type = other RNA
gtaggttcactcctgtgttcctac

SEQ ID NO: 51 - RNA, 20 nt, synthetic construct
  source 1..20: mol_type = other RNA
tggatcaccatggactacca

SEQ ID NO: 52 - DNA, 52 bp, synthetic construct
  source 1..52: mol_type = other DNA
acactctttccctacacgacgctcttccgatctttttttttttttttttttt

SEQ ID NO: 53 - DNA, 49 bp, synthetic construct
  source 1..49: mol_type = other DNA
aaaaaaaaaaaaaaaaaaaaaaaaaaagatcggaagagcgtcgtgtagg

SEQ ID NO: 54 - DNA, 62 bp, synthetic construct
  source 1..62: mol_type = other DNA
gcgccacgattcaacgtggcgcaaaaaaaaaaaaaaaaaaaagatcggaagagcgtcgtgta

SEQ ID NO: 55 - DNA, 52 bp, synthetic construct
  source 1..52: mol_type = other DNA
gtgactggagttcagacgtgtgctcttccgatcccccccccccccccccccc

SEQ ID NO: 56 - DNA, 30 bp, synthetic construct
  source 1..30: mol_type = other DNA
caccgagatctacactctttccctacacga

SEQ ID NO: 57 - DNA, 28 bp, synthetic construct
  source 1..28: mol_type = other DNA
aatgatacggcgaccaccgagatctaca

SEQ ID NO: 58 - DNA, 13 bp, synthetic construct
  source 1..13: mol_type = other DNA
cggcatacgagat

SEQ ID NO: 59 - DNA, 17 bp, synthetic construct
  source 1..17: mol_type = other DNA
tgactggagttcagacg

SEQ ID NO: 60 - DNA, 22 bp, synthetic construct
  source 1..22: mol_type = other DNA
caagcagaagacggcatacgag